European Patent Application EP 4 678 654 A1, published January 14, 2026. Title: CHIMERIC PROTEIN, HOST MICROBIAL CELL, PROCESS FOR OBTAINING SAID CHIMERIC PROTEIN, LEPTOSPIROSIS SEROLOGICAL DIAGNOSIS KIT, IN VITRO METHOD FOR EARLY SEROLOGICAL DIAGNOSIS OF LEPTOSPIROSIS, AND USE OF SAID CHIMERIC PROTEIN. Applicant: INSTITUTO BUTANTAN. The sequence listing filed with the application follows.

SEQUENCE LISTING (47 sequences)

SEQ ID NO: 1 - protein, 330 aa, Leptospira interrogans
MQFSLLQFVILNVIFLEFGGFMKRYLSIVILCTFAMLLLVCSTNKSSGSDQVKTESNATSARIVWLLGDVKILSDSGEKKAELGASLSSTDRVVTGPNGGAEIMVADSGIIKMSKNSDIEISSLMNPNGSDTNVQVNYGKIVTMVKKGQKTTEFTVSTPTALAGVRGTSFLTSVESPEGSKINCAKANCTVRFAVIEGTIAVSKKGESSEVILSKNRELRIEKNQKLTDKLIRSLQNDSLSEMKELIVLHKNETFEYGKLVEELKSSSEELKILSQSGSVEEVKAAFQKREADRNNADEITKTAKAVNETKYVQQDVQKEKLKLNPKETF

SEQ ID NO: 2 - protein, 60 aa, synthetic construct
  REGION 1..60: note = LIC10123 protein specific region
TNVQVNYGKIVTMVKKGQKTTEFTVSTPTALAGVRGTSFLTSVESPEGSKINCAKANCTV

SEQ ID NO: 3 - protein, 231 aa, Leptospira interrogans
MKFSIIKNLNLVLALLVLSSCKDDRIKISDLGVIDKDKKNQTAFVLQPEKLLVMVRTDSNLDGKTDLWTWVRGDDKDPKTSLVLFEELIRKGNHSRTWYGPGNRKLIEQSDLDENGTWESMVYYNAFAVPKETMRIVAHVEVDLYGKGKPSLWIFPEARMELDSNEDGKPDQILTNQDRMLENFTQLQKGKQIQEKDFSPMPANSSWVLNPNQITNPRYQALIRQSLFPVN

SEQ ID NO: 4 - protein, 75 aa, synthetic construct
  REGION 1..75: note = LIC13059 specific region
KDPKTSLVLFEELIRKGNHSRTWYGPGNRKLIEQSDLDENGTWESMVYYNAFAVPKETMRIVAHVEVDLYGKGKP

SEQ ID NO: 5 - protein, 366 aa, Leptospira interrogans
MKGSTLVRLAIALFMFVNVVLFAQEDLDESSTPQANTQGQSGSSTPAKTSQNSGTTQGEEVKKADLYVNSKSSFEISAQDDSSTVDYIEYKIGEMDYAKYTSPITILKEGVNRLTYRAVDKAGNKEPAKALVVVVDNTAPTVKIVPSEILYNLDGYNFGSKNVTYTISAIDALSGVKEIKYSINGGDMRSYDNQPIKLEKAGVNLIKYSAVDNSGNSSSEAILVVTLDDVKPEVEIQGNTPLVIIDGKTYSRKGNSFAIKAVDGQSGIKRILIKLDKNSDFVPYAEPITIDAQGEHTIEAKAIDNVGNESETKKVSFAVDVNPPTTQIRKVEVGTNNGSQSTSESKPAPAPAAPAAKPTTTQPTKK

SEQ ID NO: 6 - protein, 40 aa, synthetic construct
  REGION 1..40: note = LIC13050 protein specific region
TSPITILKEGVNRLTYRAVDKAGNKEPAKALVVVVDNTAP

SEQ ID NO: 7 - protein, 37 aa, synthetic construct
  REGION 1..37: note = LIC13050 protein specific region 2
ITIDAQGEHTIEAKAIDNVGNESETKKVSFAVDVNPP

SEQ ID NO: 8 - protein, 459 aa, Leptospira interrogans
MSAQTVSKIEPISINLFLRNTPVSQMGFGLPLILGVKEPTYSLQVSGNSGGLIWKSTHTGIVFIQIKYVVSGNNTSLSVVRTGTGTENDPYIISVNVSTDANGVATSTAHQIKLAAESISNIAGATKIVDVIEVANSGSGIVSAFAQTALGYERYMEISSSDDLLELGFISSDKEYIQAAQMFRQTPRPKRVAVFLLTSWSAASTEISALRNSGKDSWFKTIATTHDKETIHALGDYLASIEKMFFACSDDLSVLTGRNSIWEYITLHKTPNSFPEAAWVGNSAPRRVGSYNYAYLPLDGVENSGYANSQVSSVFAENGNLIVDFGGKQVPYPGISTGNVYADVVENRSWLKARLKENISSLFLNSDVVPYTIQGIQMIEAKMREVFVQAGIQGIIAPVETDTDKTRSDLGDYQYKINLPDTIDEIPTNDRNNRVLPNVTFSCRLRGAINEVDIDGELT

SEQ ID NO: 9 - protein, 86 aa, synthetic construct
  REGION 1..86: note = LIC12615 protein specific region
SNIAGATKIVDVIEVANSGSGIVSAFAQTALGYERYMEISSSDDLLELGFISSDKEYIQAAQMFRQTPRPKRVAVFLLTSWSAAST

SEQ ID NO: 10 - protein, 224 aa, Leptospira interrogans
MNIEIISKPSYSFAKVLLNGGESIKAESGSMMSMSSGITIQTHKAQQGGFFKSLKVAFLGGESFWMNTFTASSGNGEVLLAPTLPGDVERIELSGTVYVQSSSFLASSPNIEMDTKFQGLKGFISGESLFFLRLSGNGFLLISSYGGIDVLNVDGEMIVDTGHIVAFEEGLNYEMTKFGGWKSFFLGGEGFVARFKGKGKVWIQSRNVPSLGSWFRNQLPPIKR

SEQ ID NO: 11 - protein, 86 aa, synthetic construct
  REGION 1..86: note = LIC11636 protein specific region
TASSGNGEVLLAPTLPGDVERIELSGTVYVQSSSFLASSPNIEMDTKFQGLKGFISGESLFFLRLSGNGFLLISSYGGIDVLNVDG

SEQ ID NO: 12 - protein, 272 aa, Leptospira interrogans
MKKLSILAISVALFASITACGAFGGLPSLKSSFVLSEDTIPGTNETVKTLLPYGSVINYYGYVKPGQAPDGLVDGNKKAYYLYVWIPAVIAEMGVRMISPTGEIGEPGDGDLVSDAFKAATPEEKSMPHWFDTWIRVERMSAIMPDQIAKAAKAKPVQKLDDDDDGDDTYKEERHNKYNSLTRIKIPNPPKSFDDLKNIDTKKLLVRGLYRISFTTYKPGEVKGSFVASVGLLFPPGIPGVSPLIHSNPEELQKQAIAAEESLKKAASDATK

SEQ ID NO: 13 - protein, 31 aa, synthetic construct
  REGION 1..31: note = LIC11352 protein specific region 1
GDGDLVSDAFKAATPEEKSMPHWFDTWIRVE

SEQ ID NO: 14 - protein, 53 aa, synthetic construct
  REGION 1..53: note = LIC11352 protein specific region 2
GEVKGSFVASVGLLFPPGIPGVSPLIHSNPEELQKQAIAAEESLKKAASDATK

SEQ ID NO: 15 - protein, 202 aa, Leptospira interrogans
MGVTMIRLLIVFLVLVFFNVCKPKTAESSDAVVTFLRGKASVIETGKELSTYTNVTEKQSVKTESEAVLDLTSKLGSFRLLGGSTATIAALNSESASFQVSEGNVLIKAGNLAKGQSLIVHTPTVVAAVRGTQFWGRVNGKDETGTFAVREGAVEITRKSDNAKVLIEAGQALDLKPGDRDLKVRVAAKEELAAMEQIDQMK

SEQ ID NO: 16 - protein, 72 aa, synthetic construct
  REGION 1..72: note = LIC11122 protein specific region
STATIAALNSESASFQVSEGNVLIKAGNLAKGQSLIVHTPTVVAAVRGTQFWGRVNGKDETGTFAVREGAVE

SEQ ID NO: 17 - protein, 315 aa, Leptospira interrogans
MTKKVLVLGSIVLFCFSLIHCSPNKNNNDSELLSLAALIALGNQGIQFSAYAGSQKLECGQTLRGHSRSLETISFIPNAHIAESTTFQLHDFRLFVHGVTLIQNSGEETPLTLNQDGKFQSGEIALLDFENKTGKCNGTTDTNNVVSALIPSGTYQGIKFIVGIPENKNHLDADNQSPPLDNSGMFWSWTSGYKFLKLDFETAETLGVETSVHIGSANCVGSGSSSTCARVNRIPVTLIPEGGFNPSTQEIKINIQALLQGIDLTANPNAAMCMSGLVGATSTGCPTIFANIGLDLNAGTPITPAKTVFSIKAKN

SEQ ID NO: 18 - protein, 76 aa, synthetic construct
  REGION 1..76: note = LIC11089 protein specific region 2
SELLSLAALIALGNQGIQFSAYAGSQKLECGQTLRGHSRSLETISFIPNAHIAESTTFQLHDFRLFVHGVTLIQNS

SEQ ID NO: 19 - protein, 440 aa, Leptospira interrogans
MNLKKITHYLLLWIVVSFLFSNCKSEANNDSERLALLMTLFQPTATRAQVVDRYLQLGYESYDQSYKDAVAFQTAVTAFAANNNPTAADHINLKNLYVVARASYLTTEAFRFSSGPIDNVDILGCGSNADGSGDEECEGLINGWPLDESAIDNYINNNAAQQPTYAAILAANGDAGANNAVDQDDETALTVGWHAIEYILWGQDLFNGGINQISGQRNIADLTGASPGTVGGRRRTYMKAVTDGLVLQLKLIRDQFEDGARYSDGLKSNPDAAVTYIFQGLGKFIAGEWGGERLTGTFGGQQEEEHSCFSDTTKADFYYNAQSVLNIWNGSYELKKGTVTSTGPGLKNLFGTFNVPGIGFQATAARDTFCINLSEQTADPNYTTSCKPGSLTGRYDQIIRNTDNEYQILFDVQKFIGDKMKKTITDAAKTIGISITDFSI

SEQ ID NO: 20 - protein, 43 aa, synthetic construct
  REGION 1..43: note = LIC10713 protein specific region
QQPTYAAILAANGDAGANNAVDQDDETALTVGWHAIEYILWGQ

SEQ ID NO: 21 - protein, 480 aa, Leptospira interrogans
MLKKSSALILVFCFLAWGCSFNKGKDDNSKNLELLLGLYLLNEANYYCAPEENVRTSGSAPNFSISTSNLSQVLLTENGVYADGGTAYLVGTVEFPGIGRNNPLGIVYAEQNHQFASNSNRFIYPLWINKSGDLIQDDQKSESPGYRSTTTAFPIGSTPGYYAPSADYNNFNSNLLGTTFVVPANLSTPVITKKVTNNTPQTCEEYKFRTEQNGLLGSSSSGLSKVWQSRKKLNINLIFIPGAVATPTVAGMATMIQTLKDIYAQNTVKIDVTVTASIAAAGAPYLTIQNITDDYGDVANSLGNLYKTNPNNAQDSNSLNIYITRDYTVSNDAPAGILGISSGIPGIPVTGTPRSGMIVFIENHRTASGCGVQGQDLICASDQVFLAKTIAHEGGHYLGLYHLVEKDVIKGRYSLDPLPETPECKDQNGNNIVGLTECLGEGFYNSGGLNLMFWAGNPKIDQTQLTGEQGWVLRSHPLVY

SEQ ID NO: 22 - protein, 91 aa, synthetic construct
  REGION 1..91: note = LIC13434 protein specific region
GQDLICASDQVFLAKTIAHEGGHYLGLYHLVEKDVIKGRYSLDPLPETPECKDQNGNNIVGLTECLGEGFYNSGGLNLMFWAGNPKIDQTQ

SEQ ID NO: 23 - protein, 15 aa, synthetic construct
  REGION 1..15: note = Linker
GGGGSGGGGSGGGGS

SEQ ID NO: 24 - protein, 915 aa, synthetic construct
  REGION 1..915: note = Chimeric protein
TNVQVNYGKIVTMVKKGQKTTEFTVSTPTALAGVRGTSFLTSVESPEGSKINCAKANCTVGGGGSGGGGSGGGGSKDPKTSLVLFEELIRKGNHSRTWYGPGNRKLIEQSDLDENGTWESMVYYNAFAVPKETMRIVAHVEVDLYGKGKPGGGGSGGGGSGGGGSTSPITILKEGVNRLTYRAVDKAGNKEPAKALVVVVDNTAPGGGGSGGGGSGGGGSITIDAQGEHTIEAKAIDNVGNESETKKVSFAVDVNPPGGGGSGGGGSGGGGSSNIAGATKIVDVIEVANSGSGIVSAFAQTALGYERYMEISSSDDLLELGFISSDKEYIQAAQMFRQTPRPKRVAVFLLTSWSAASTGGGGSGGGGSGGGGSTASSGNGEVLLAPTLPGDVERIELSGTVYVQSSSFLASSPNIEMDTKFQGLKGFISGESLFFLRLSGNGFLLISSYGGIDVLNVDGGGGGSGGGGSGGGGSGDGDLVSDAFKAATPEEKSMPHWFDTWIRVEGGGGSGGGGSGGGGSGEVKGSFVASVGLLFPPGIPGVSPLIHSNPEELQKQAIAAEESLKKAASDATKGGGGSGGGGSGGGGSSTATIAALNSESASFQVSEGNVLIKAGNLAKGQSLIVHTPTVVAAVRGTQFWGRVNGKDETGTFAVREGAVEGGGGSGGGGSGGGGSSELLSLAALIALGNQGIQFSAYAGSQKLECGQTLRGHSRSLETISFIPNAHIAESTTFQLHDFRLFVHGVTLIQNSGGGGSGGGGSGGGGSQQPTYAAILAANGDAGANNAVDQDDETALTVGWHAIEYILWGQGGGGSGGGGSGGGGSGQDLICASDQVFLAKTIAHEGGHYLGLYHLVEKDVIKGRYSLDPLPETPECKDQNGNNIVGLTECLGEGFYNSGGLNLMFWAGNPKIDQTQ

SEQ ID NO: 25 - DNA, 2760 bp, synthetic construct
  misc_feature 1..2760: note = Chimeric gene
  source 1..2760: mol_type = other DNA
ctcgagaccaacgtgcaggtgaactatggcaaaattgtgaccatggtgaaaaaaggccagaaaaccaccgaatttaccgtgagcaccccgaccgcgctggcgggcgtgcgcggcaccagctttctgaccagcgtggaaagcccggaaggcagcaaaattaactgcgcgaaagcgaactgcaccgtgggcggcggcggcagcggcggcggcggcagcggcggcggcggcagcaaagatccgaaaaccagcctggtgctgtttgaagaactgattcgcaaaggcaaccatagccgcacctggtatggcccgggcaaccgcaaactgattgaacagagcgatctggatgaaaacggcacctgggaaagcatggtgtattataacgcgtttgcggtgccgaaagaaaccatgcgcattgtggcgcatgtggaagtggatctgtatggcaaaggcaaaccgggcggcggcggcagcggcggcggcggcagcggcggcggcggcagcaccagcccgattaccattctgaaagaaggcgtgaaccgcctgacctatcgcgcggtggataaagcgggcaacaaagaaccggcgaaagcgctggtggtggtggtggataacaccgcgccgggcggcggcggcagcggcggcggcggcagcggcggcggcggcagcattaccattgatgcgcagggcgaacataccattgaagcgaaagcgattgataacgtgggcaacgaaagcgaaaccaaaaaagtgagctttgcggtggatgtgaacccgccgggcggcggcggcagcggcggcggcggcagcggcggcggcggcagcagcaacattgcgggcgcgaccaaaattgtggatgtgattgaagtggcgaacagcggcagcggcattgtgagcgcgtttgcgcagaccgcgctgggctatgaacgctatatggaaattagcagcagcgatgatctgctggaactgggctttattagcagcgataaagaatatattcaggcggcgcagatgtttcgccagaccccgcgcccgaaacgcgtggcggtgtttctgctgaccagctggagcgcggcgagcaccggcggcggcggcagcggcggcggcggcagcggcggcggcggcagcaccgcgagcagcggcaacggcgaagtgctgctggcgccgaccctgccgggcgatgtggaacgcattgaactgagcggcaccgtgtatgtgcagagcagcagctttctggcgagcagcccgaacattgaaatggataccaaatttcagggcctgaaaggctttattagcggcgaaagcctgttttttctgcgcctgagcggcaacggctttctgctgattagcagctatggcggcattgatgtgctgaacgtggatggcggcggcggcggcagcggcggcggcggcagcggcggcggcggcagcggcgatggcgatctggtgagcgatgcgtttaaagcggcgaccccggaagaaaaaagcatgccgcattggtttgatacctggattcgcgtggaaggcggcggcggcagcggcggcggcggcagcggcggcggcggcagcggcgaagtgaaaggcagctttgtggcgagcgtgggcctgctgtttccgccgggcattccgggcgtgagcccgctgattcatagcaacccggaagaactgcagaaacaggcgattgcggcggaagaaagcctgaaaaaagcggcgagcgatgcgaccaaaggcggcggcggcagcggcggcggcggcagcggcggcggcggcagcagcaccgcgaccattgcggcgctgaacagcgaaagcgcgagctttcaggtgagcgaaggcaacgtgctgattaaagcgggcaacctggcgaaaggccagagcctgattgtgcataccccgaccgtggtggcggcggtgcgcggcacccagttttggggccgcgtgaacggcaaagatgaaaccggcacctttgcggtgcgcgaaggcgcggtggaaggcggcggcggcagcggcggcggcggcagcggcggcggcggcagcagcgaactgctgagcctggcggcgctgattgcgctgggcaaccagggcattcagtttagcgcgtatgcgggcagccagaaactggaatgcggccagaccctgcgcggccatagccgcagcctggaaaccattagctttattccgaacgcgcatattgcggaaagcaccacctttcagctgcatgattttcgcctgtttgtgcatggcgtgaccctgattcagaacagcggcggcggcggcagcggcggcggcggcagcggcggcggcggcagccagcagccgacctatgcggcgattctggcggcgaacggcgatgcgggcgcgaacaacgcggtggatcaggatgatgaaaccgcgctgaccgtgggctggcatgcgattgaatatattctgtggggccagggcggcggcggcagcggcggcggcggcagcggcggcggcggcagcggccaggatctgatttgcgcgagcgatcaggtgtttctggcgaaaaccattgcgcatgaaggcggccattatctgggcctgtatcatctggtggaaaaagatgtgattaaaggccgctatagcctggatccgctgccggaaaccccggaatgcaaagatcagaacggcaacaacattgtgggcctgaccgaatgcctgggcgaaggcttttataacagcggcggcctgaacctgatgttttgggcgggcaacccgaaaattgatcagacccagtaaaagctt

SEQ ID NO: 26 - DNA, 993 bp, Leptospira interrogans
  source 1..993: mol_type = genomic DNA
ttgcaattttctctcctacaatttgttattttaaatgtcatctttttagagtttgggggttttatgaaacgttatttgagtattgtgattctctgtacgtttgcgatgttattgctcgtttgtagcacgaacaaatcatccggcagcgatcaggtaaaaaccgagtctaatgctaccagcgcaagaatcgtttggcttcttggagacgtaaaaattctttccgattctggagaaaaaaaagcagagttaggtgcttctctttcttctacggaccgtgttgtaacaggaccgaacggcggagctgagattatggtcgcagacagtggaattattaagatgtctaaaaattccgatatagaaatttccagccttatgaatccaaacggttccgatacaaatgttcaagtgaactacggaaagatcgtgacgatggtaaaaaaaggtcagaaaactacagagtttaccgtttctactccgactgcacttgcaggtgttaggggaacttccttcctaacttctgtagaaagtccagaaggatctaagattaattgtgccaaagccaattgtaccgttcgttttgcagtgatcgaagggaccattgcagtttctaaaaagggagaatcttccgaagtaattctgagtaaaaaccgcgagctcagaattgaaaagaatcaaaaactcaccgacaaactgattcgttcacttcaaaacgattctctttccgaaatgaaagaactcatcgttcttcataaaaacgaaactttcgaatacggaaaattagtagaagaacttaaatcttccagcgaagaactcaaaattttgagccaatctggttctgtggaagaagtaaaagctgcgtttcaaaaaagagaagcggatcgtaataacgcggacgagattacaaaaaccgctaaggcagtaaacgaaaccaaatatgtacaacaagatgtacaaaaggaaaaactgaaattgaatccaaaagaaacattttag

SEQ ID NO: 27 - DNA, 180 bp, synthetic construct
  misc_feature 1..180: note = Nucleotide sequence encoding the specific region of the LIC10123 protein
  source 1..180: mol_type = other DNA
accaatgtccaggtgaactatggtaaaattgtgaccatggtgaaaaaaggccagaaaaccaccgaatttaccgttagcaccccgaccgcactggcaggcgttcgtggcaccagctttctgaccagcgttgaaagtccggaaggtagcaaaattaactgtgcaaaagcaaattgtaccgtg

SEQ ID NO: 28 - DNA, 696 bp, Leptospira interrogans
  source 1..696: mol_type = genomic DNA
atgaaattcagtataatcaaaaatttgaatttagtacttgccctactcgttttatcttcttgcaaagatgatagaattaaaataagcgatctaggtgtaatcgacaaagataaaaaaaatcaaacagcctttgttcttcaaccggaaaaactactcgtgatggtgcgaaccgattcgaatctggatggaaaaacggatctatggacttgggtacgcggagacgataaggatcctaaaacaagtttggttttatttgaagaactcattcgaaaaggaaatcatagtcggacttggtatggtccaggaaatcgaaaattaatcgaacaaagtgatttagacgaaaatggaacttgggaatccatggtatattataacgcatttgcagttcccaaagaaacaatgagaattgtagcacatgtagaagtagatctttatggaaaaggcaaaccaagtttatggattttcccggaagctcgaatggaattagattcaaacgaagacggaaaaccggatcaaatattgaccaatcaagatcgtatgttagaaaattttacccaacttcaaaaaggaaaacaaattcaagagaaggattttagtccgatgcctgcaaacagttcttgggtattaaacccgaaccaaattacaaaccctcggtatcaggcattgattcgtcaaagtctttttccagtaaattaa

SEQ ID NO: 29 - DNA, 225 bp, synthetic construct
  misc_feature 1..225: note = Nucleotide sequence encoding the specific region of the LIC13059 protein
  source 1..225: mol_type = other DNA
aaagatccgaaaaccagcctggttctgtttgaagaactgattcgtaaaggtaatcatagccgtacctggtatggtccgggtaatcgtaaactgattgaacagagcgatctggatgaaaatggcacctgggaaagcatggtgtattataacgcatttgcagttccgaaagaaaccatgcgtattgttgcacatgttgaggttgatctgtatggtaaaggcaaaccg

SEQ ID NO: 30 - DNA, 1101 bp, Leptospira interrogans
  source 1..1101: mol_type = genomic DNA
atgaagggttctactctcgtacgactcgcaatcgctttattcatgtttgttaacgtagtgctttttgcccaggaagatctggatgaaagctctactcctcaggcaaatactcaaggacaatccgggagttccactcctgcaaaaacttcccaaaattctggaactactcagggagaagaagttaaaaaagcggatctttatgtgaactcaaaaagttcttttgaaatttccgcccaagacgactccagcacggtcgattatatcgaatataaaatcggcgaaatggactacgcaaaatatacttctccaatcacaattctaaaagaaggcgttaaccgacttacttatagagccgtggataaagccggaaacaaagaacctgctaaagcgctcgtcgtcgttgtggataataccgctccgactgtaaaaattgttccgagtgaaattctttataatttggacggctataacttcggttccaaaaacgtaacctatacaatctctgcgatcgacgctctttccggtgtcaaagaaattaaatattccatcaacggtggagacatgagatcctatgataaccagcctattaaattagaaaaggctggagtgaatttgattaaatactccgctgtggataattctggaaactcttcttccgaggcaattcttgtagtaaccttggatgacgtaaaaccggaagttgaaatccaagggaacactcctctggtaatcatcgatgggaaaacatattccagaaaaggaaactcatttgcaatcaaagcggtcgacggacaatccggaattaaaagaattctaattaaattggataaaaattcagatttcgttccttacgcagagcctatcacgatcgatgctcaaggtgaacatacaatcgaagccaaagcgattgacaacgtaggaaacgaaagtgagaccaaaaaggtcagttttgcagtagatgtaaatccacctacaacacaaattcgtaaagtagaagtaggaacaaacaatggaagccaatctacttccgaatcaaaacctgctcccgctccggcggctcctgcagcgaaacctactactactcaacctacaaaaaaataa

SEQ ID NO: 31 - DNA, 120 bp, synthetic construct
  misc_feature 1..120: note = Nucleotide sequence encoding specific region 1 of the LIC13050 protein
  source 1..120: mol_type = other DNA
accagcccgattaccattctgaaagaaggtgttaatcgtctgacctatcgtgcagttgataaagccggtaataaagaaccggcaaaagcactggttgttgttgtggataataccgcacca

SEQ ID NO: 32 - skipped

SEQ ID NO: 33 - DNA, 1380 bp, Leptospira interrogans
  source 1..1380: mol_type = genomic DNA
atgagcgcacaaacagtctctaaaatagaaccgatcagtattaatctatttcttaggaatactccggtttctcaaatgggattcggattacctttgattttaggagttaaagagccgacctattctttacaagtttccggaaattccggcggacttatttggaagtctacacatactggaattgtatttatacaaattaaatacgtggtttcaggaaacaacactagtcttagtgtcgtccgtactggaaccggtacagaaaacgatccttatataatttcggttaatgtttctacggatgcaaacggagtggctacgtctaccgcgcatcaaatcaaattagcagctgagtcaatttcaaatatcgcgggagcaactaagattgtagatgtaatcgaagtggcaaattctggcagcggaattgtttccgcgtttgcacaaaccgctttgggttacgaaagatatatggaaatttcttcatcggatgatcttttggaattaggttttatttcttccgataaagaatacattcaagccgcgcagatgttcagacaaacccctagaccaaaacgggtcgcggtatttctgcttacttcctggtcggctgcttcgaccgaaatttcagctcttagaaattctggtaaagactcttggtttaaaactatagcaactactcacgataaggaaaccatacacgcgttaggtgattatctcgcttctatcgaaaaaatgttttttgcgtgttctgacgatttaagcgttttaactggaagaaattctatctgggagtacatcactcttcataaaactccaaattcttttccggaagccgcttgggtaggaaattctgctcctcgcagagtcggttcgtataactacgcttatttgcctttggatggagtggaaaattcgggttatgcgaattcacaggtaagttccgtatttgcggaaaatggaaatttgatcgtagatttcggaggaaaacaagttccttatccaggaatttccactgggaacgtctacgccgatgtagtcgaaaatcgctcttggctcaaagctcgtctgaaagaaaacatctcaagtctttttctgaactcggatgttgtaccttatacaattcaaggaattcagatgattgaagcgaagatgcgtgaagtttttgttcaagctggaattcaaggtatcatcgcgccggtggaaacggatacggataaaacacgttctgatcttggcgattatcaatataaaatcaatttaccagatacgatagacgaaattccgacaaatgatcggaacaaccgtgttcttcctaacgtcactttttcgtgccgtttaagaggagcgatcaacgaagtcgacatagacggggaattaacctaa

SEQ ID NO: 34 - DNA, 258 bp, synthetic construct
  misc_feature 1..258: note = Nucleotide sequence encoding the specific region of the LIC12615 protein
  source 1..258: mol_type = other DNA
agtaatattgccggtgcaaccaaaattgtggatgttattgaagttgcaaatagcggtagcggtattgttagcgcatttgcccagacagcactgggttatgaacgttatatggaaattagcagcagtgatgatctgctggaactgggttttattagcagcgataaagaatatatccaggcagcacagatgtttcgtcagacaccgcgtccgaaacgtgttgcagtttttctgctgaccagttggagcgcagcaagcaca

SEQ ID NO: 35 - DNA, 675 bp, Leptospira interrogans
  source 1..675: mol_type = genomic DNA
atgaatattgaaattattagcaaaccgtcttatagttttgcaaaggttcttttaaatggaggagaatcgatcaaagcggaatccggttctatgatgtctatgagttctggaattacgattcaaactcataaagcacaacaaggcggattttttaaaagtttaaaagtagcttttttaggcggagaatctttttggatgaatacttttactgcttcttctggaaacggagaagtattactcgcaccaactcttccgggagacgtggaaagaatagaattatctggaacggtttatgtacagtccagttcttttcttgcatcttcaccgaacattgaaatggatacaaagtttcaaggactcaaagggtttatcagtggagaatctctattttttcttagactttcaggaaacggttttcttttaatttcgagttacggtggaatagacgttttaaacgtagacggagaaatgatcgtagacactggacatatcgtagcctttgaagaaggtttaaactacgagatgactaagtttgggggttggaagtctttctttttaggtggagagggatttgtggcccgttttaaaggaaaaggaaaggtttggattcagtctagaaacgttccttctttaggaagttggtttagaaaccaacttcctccgattaaaagataa

SEQ ID NO: 36 - DNA, 258 bp, synthetic construct
  misc_feature 1..258: note = Nucleotide sequence encoding the specific region of the LIC11636 protein
  source 1..258: mol_type = other DNA
accgcaagcagcggtaatggtgaagttctgctggcaccgaccctgcctggtgatgttgaacgtattgaactgagcggcaccgtttatgttcagagcagctcatttctggcaagcagcccgaatattgaaatggataccaaatttcagggtctgaaaggctttattagcggtgaaagcctgttttttctgcgtctgagtggtaacggtttcctgctgattagcagctatggtggtattgatgttctgaatgttgatggt

SEQ ID NO: 37 - DNA, 819 bp, Leptospira interrogans
  source 1..819: mol_type = genomic DNA
atgaaaaaactttcgattttggctatctccgttgcactctttgcaagcattaccgcttgtggtgctttcggtggtctgccaagcctaaaaagctcttttgttctgagcgaggacacaatcccagggacaaacgaaaccgtaaaaacgttacttccctacggatctgtgatcaactattacggatacgtaaagccaggacaagcgccggacggtttagtcgatggaaacaaaaaagcatactatctctatgtttggattcctgccgtaatcgctgaaatgggagttcgtatgatttccccaacaggcgaaatcggtgagccaggcgacggagacttagtaagcgacgctttcaaagcggctaccccagaagaaaaatcaatgccacattggtttgatacttggatccgtgtagaaagaatgtcggcgattatgcctgaccaaatcgccaaagctgcgaaagcaaaaccagttcaaaaattggacgatgatgatgatggtgacgatacttataaagaagagagacacaacaagtacaactctcttactagaatcaagatccctaatcctccaaaatcttttgacgatctgaaaaacatcgacactaaaaaacttttagtaagaggtctttacagaatttctttcactacctacaaaccaggtgaagtgaaaggatctttcgttgcatctgttggtctgcttttcccaccaggtattccaggtgtgagcccgctgatccactcaaatcctgaagaattgcaaaaacaagctatcgctgctgaagagtctttgaaaaaagctgcttctgacgcgactaagtaa

SEQ ID NO: 38 - DNA, 93 bp, synthetic construct
  misc_feature 1..93: note = Nucleotide sequence encoding the specific region 1 of the LIC1135 protein
  source 1..93: mol_type = other DNA
ggtgatggtgatctggttagtgatgcatttaaagcagcaacaccggaagaaaaaagcatgccgcattggtttgatacctggattcgtgttgaa

SEQ ID NO: 39 - DNA, 159 bp, synthetic construct
  misc_feature 1..159: note = Nucleotide sequence encoding the specific region 2 of the LIC11352 protein
  source 1..159: mol_type = other DNA
ggcgaagttaaaggtagctttgttgcaagcgttggtctgctgtttccgcctggtattccgggtgttagtccgctgattcatagcaatccggaagaactgcagaaacaggcaattgcagcagaagaaagcctgaaaaaagccgcaagtgatgccaccaaa

SEQ ID NO: 40 - DNA, 609 bp, Leptospira interrogans
  source 1..609: mol_type = genomic DNA
atgggagttactatgattcgattattaattgtgtttttggttttagtctttttcaacgtttgtaaacctaagaccgccgaaagttcagatgcagtagtcacttttctcagaggaaaagcttccgtcatagaaacgggtaaagagctttctacttatacaaacgtaactgaaaaacaatctgtaaaaaccgagtcggaggctgtactagatctcacttctaaattagggagttttcgtctattaggaggaagtactgcaaccatagcagctcttaattctgagagtgcttcgttccaagtttccgaaggaaacgtattgatcaaggcgggtaatcttgcaaaaggacagagccttattgtgcatactcctactgtagttgcagctgttcgaggaacccagttttggggaagagtgaacggtaaagacgagacaggaacttttgcggttcgagaaggagccgttgaaattactcgcaaatctgacaatgcaaaagttttaattgaagcaggtcaggccttggatctcaaaccgggtgatagggacttaaaagtaagagttgcagccaaagaagaattagcagcgatggagcagattgaccaaatgaaatga

SEQ ID NO: 41 - DNA, 216 bp, synthetic construct
  misc_feature 1..216: note = Nucleotide sequence encoding the specific region of the LIC11122 protein
  source 1..216: mol_type = other DNA
agcaccgcaaccattgcagcactgaatagcgaaagcgcaagctttcaggttagcgaaggtaatgttctgattaaagcaggtaatctggcaaaaggtcagagcctgattgttcataccccgacagttgttgcagcagttcgtggtacacagttttggggtcgtgttaatggtaaagatgaaaccggcacctttgcggttcgtgaaggtgccgttgag

SEQ ID NO: 42 - DNA, 948 bp, Leptospira interrogans
  source 1..948: mol_type = genomic DNA
atgactaaaaaagttttagtcttaggttctatcgttttattttgtttttctttgattcattgttctccaaataaaaataataatgattccgaattgttatcattagctgctttgatcgcactcggaaatcaaggaattcagttttccgcttacgccggttctcaaaaattagaatgtggtcaaaccctcagaggtcattctagatctttagaaacgatctccttcattcccaatgcacacattgcagagagcactacgtttcaattacacgactttcgtctttttgtacacggagttactttgatccaaaactctggagaagaaactcctctcactctcaatcaagacggtaagtttcaatccggagaaatcgctcttttagattttgaaaataaaacaggaaagtgtaatggtactacggatacaaataacgtcgtttctgcgttaattccttcgggtacgtatcaaggtattaagtttatcgtcgggatacctgaaaacaaaaatcacttagatgcagacaatcaatctcccccactcgataactctggaatgttctggagttggacaagcggttataagtttttaaagctggattttgaaaccgccgaaaccttaggcgtagaaacttcggtccacataggttctgccaattgtgtaggctctggaagttcgagtacttgcgcgagagtcaatcgtattccggtcaccctaattccggaaggtggttttaatccttccactcaagaaattaaaatcaacattcaagctcttttacaaggaattgatcttaccgccaacccaaacgcagcgatgtgtatgtcaggacttgtaggcgcaacaagcaccggttgtcctaccatctttgcaaacataggtttggatctaaatgcaggcaccccgattactccggccaaaaccgttttttcgatcaaggctaaaaattaa

SEQ ID NO: 43 - DNA, 228 bp, synthetic construct
  misc_feature 1..228: note = Nucleotide sequence encoding the specific region of the LIC11089 protein
  source 1..228: mol_type = other DNA
agtgaactgctgagcctggcagccctgattgcactgggtaatcagggtattcagtttagcgcatatgcaggtagccagaaactggaatgtggccagaccctgcgtggtcatagtcgtagcctggaaaccattagctttattccgaatgcacatattgcagaaagtaccacctttcagctgcatgattttcgtctgtttgttcatggtgtgaccctgattcagaatagt

SEQ ID NO: 44 - DNA, 1323 bp, Leptospira interrogans
  source 1..1323: mol_type = genomic DNA
atgaatctaaaaaaaatcacacactatcttctactttggatcgttgtatcgtttcttttctcaaattgtaaatcagaagcaaacaacgactcagaacgtttagccttattgatgactttattccaacccactgcgacaagagctcaagtcgtagatcgttatcttcaactcggctacgaatcctacgatcagagttataaagacgcagtcgcttttcagaccgcagttacagcctttgccgccaataacaacccgaccgcagcggatcatatcaatcttaaaaatttatacgtagtagcaagagcttcttatttaactacggaagcatttcgtttttcatctggaccgatagacaacgtagacattttaggttgcggaagtaatgcggatggttccggagacgaagaatgcgaaggactgatcaacggatggccgttagacgaaagtgcgattgataattatattaataacaatgctgcacaacaaccaacctacgcagccatcttagctgcaaacggagatgcaggtgcaaataacgcagttgatcaagacgatgagacagcgcttacagtcggttggcacgccatcgaatatatactctggggtcaggatctatttaacggaggaatcaatcaaatttcaggacaacgtaatatagctgatcttacaggagcttctccaggaacagttggaggcagaagaagaacttatatgaaagcagttacggacggactggttcttcagctaaaattgattcgagatcaatttgaagacggtgccagatattcggatggacttaaatccaatcctgacgcagcggtcacttatatctttcaaggacttggtaaattcatcgctggcgaatggggaggagaaagacttaccggaacttttggtggacaacaagaagaagaacattcttgttttagcgatactacaaaagctgacttctattacaacgcacaaagtgtgttgaacatttggaacggatcttacgaattgaaaaaaggaaccgtaacttccacgggtccgggtttaaaaaatctttttggtacttttaacgttcctggaatcggttttcaagcgactgcagccagagacacattctgtatcaatctttcggaacaaaccgcagatccaaattatactacctcttgtaaaccaggttctttgaccggaagatacgatcaaattatcagaaacacggataacgaatatcaaatcctttttgacgtgcaaaagtttattggagacaaaatgaaaaagacgatcaccgatgccgcaaaaactataggaatttctatcacggacttttcaatttaa

SEQ ID NO: 45 - DNA, 129 bp, synthetic construct
  misc_feature 1..129: note = Nucleotide sequence encoding the specific region of the LIC10713 protein
  source 1..129: mol_type = other DNA
cagcagccgacctatgcagcaattctggcagcaaatggtgatgcgggtgcaaataatgcggttgatcaggatgatgaaacagcactgaccgttggttggcatgcaattgagtatattctgtggggtcag

SEQ ID NO: 46 - DNA, 1443 bp, Leptospira interrogans
  source 1..1443: mol_type = genomic DNA
atgttaaaaaaatcctcggctttaattttagttttttgttttcttgcatggggttgttctttcaataaaggcaaagacgataattctaaaaacttagaacttcttttaggattgtatttactcaacgaagcaaattactattgcgccccagaagaaaacgttcgaacaagcggaagcgcaccaaattttagcatatctacttctaatctcagtcaagtccttttaacagaaaacggagtatacgcggatggtggaacggcatatctagtaggtacggtagagtttcccggaattggtagaaacaatccgttaggaatcgtttatgccgaacaaaatcatcaatttgcatccaactcaaatcgttttatatatcctttatggataaataagtctggagatctaattcaagacgatcaaaagagcgaatcacccggatacagatctaccacaaccgcttttcccataggctcaactcctggctactatgcacctagtgccgattataataactttaacagtaatctattaggaacaacttttgttgttccagctaatttaagtacaccagttataactaaaaaagttacgaacaacacacctcaaacttgcgaagagtataaatttcgcactgaacaaaacggtttattaggaagttcctcttcaggtttaagtaaagtttggcaatccagaaaaaaactgaatatcaacttaatctttattccaggggcagtagccactcctaccgttgcaggtatggccacgatgattcaaacattaaaagatatttatgctcaaaacacagtaaaaatcgacgtgaccgtgacggcttccatagcagcagcaggtgcgccttatttaacaattcaaaatatcacggacgactatggagacgttgctaattcattaggaaatctttataaaacaaatcccaataacgcacaagattcaaattctttgaatatatacattacaagagattatacggtttcaaacgatgcgcccgctggaattttagggatttcctccggcatacctggaattccagttacaggtacacctagatctggtatgatcgtatttatagaaaatcatagaactgcttccggatgtggagtacaaggacaagatttgatctgtgcatcagatcaagtttttctcgcaaaaacaatcgctcatgaaggcggccattatttgggtctttatcatctagtcgaaaaagacgtaatcaaaggacgttattccttagaccctttaccagaaactccggaatgtaaagatcaaaatggaaataatatcgtaggtttaacggaatgtttaggagaaggattttacaacagcggaggattaaatctaatgttttgggcgggaaatcctaaaatcgatcaaactcaattgacaggggaacaaggttgggtgctccgttctcaccctcttgtatattaa

SEQ ID NO: 47 - DNA, 273 bp, synthetic construct
  misc_feature 1..273: note = Nucleotide sequence encoding the specific region of the LIC13434 protein
  source 1..273: mol_type = other DNA
ggtcaggatctgatttgtgcaagcgatcaggtttttctggcgaaaaccattgcccatgaaggtggtcattatctgggtctgtatcatctggttgaaaaagatgtgatcaaaggtcgttatagcctggatccgctgccggaaactccggaatgtaaagatcagaatggcaataacattgtgggtctgaccgaatgtctgggtgaaggcttttataacagcggtggtctgaatctgatgttttgggcaggcaatccgaaaattgatcagacacag